European Patent Specification EP 4 308 723 B1, published April 23, 2025. Title: TARGETED NEXT-GENERATION SEQUENCING VIA ANCHORED PRIMER EXTENSION. Applicant: F. Hoffmann-La Roche AG ROCHE SEQUENCING SOLUTIONS, INC. Roche Diagnostics GmbH. The sequence listing filed with the application follows.

SEQUENCE LISTING (11 sequences)

SEQ ID NO: 1 - DNA, 60 bp, Artificial Sequence
  Synthetic
agatcggaagagcacatccgacggtagtgtacagacagacgccgaacgattagctcttca

SEQ ID NO: 2 - DNA, 61 bp, Artificial Sequence
  Synthetic
agatcggaagagcacatccgacggtagtgtacagacagacagttatggcggaaaggtatgc

SEQ ID NO: 3 - DNA, 60 bp, Artificial Sequence
  Synthetic
agatcggaagagcacatccgacggtagtgtacagacagacaaaagaagtcagctgcgtcg

SEQ ID NO: 4 - DNA, 30 bp, Artificial Sequence
  Synthetic
agatcggaagagcacatccgactacctata

SEQ ID NO: 5 - DNA, 29 bp, Artificial Sequence
  Synthetic
actaccgtcggatgtgctcttccgatctt

SEQ ID NO: 6 - DNA, 30 bp, Artificial Sequence
  Synthetic
agatcggaagagcacatccgacggtagtgt

SEQ ID NO: 7 - DNA, 66 bp, Artificial Sequence
  Synthetic
caagcagaagacggcatacgagattcgccttagtgactggagttcagacgtgtgctcttccgatct

SEQ ID NO: 8 - DNA, 66 bp, Artificial Sequence
  Synthetic
aatgatacggcgaccaccgagatctacactagatcgctctttccctacacgatccgacggtagtgt

SEQ ID NO: 9 - DNA, 19 bp, Artificial Sequence
  Synthetic
agatcgctctttccctaca

SEQ ID NO: 10 - DNA, 2322 bp, Artificial Sequence
  Synthetic
agcttttctaatttaacctttgtcaggttaccaactactaaggttgtaggctcaagagggtgtgtcctgtcgtaggtaaataactgacctgtcgagcttaatattctatattgttgttctttctgcaaaaaagtggggaagtgagtaatgaaattatttctaacatttatctgcatcataccttccgagcatttattaagcatttcgctataagttctcgctggaagaggtagttttttcattgtactttaccttcatctctgttcattatcatcgcttttaaaacggttcgaccttctaatcctatctgaccattataattttttagaatggtttcataagaaagctctgaatcaacggactgcgataataagtggtggtatccagaatttgtcacttcaagtaaaaacacctcacgagttaaaacacctaagttctcaccgaatgtctcaatatccggacggataatatttattgcttctcttgaccgtaggactttccacatgcaggattttggaacctcttgcagtactactggggaatgagttgcaattattgctacaccattgcgtgcatcgagtaagtcgcttaatgttcgtaaaaaagcagagagcaaaggtggatgcagatgaacctctggttcatcgaataaaactaatgacttttcgccaacgacatctactaatcttgtgatagtaaataaaacaattgcatgtccagagctcattcgaagcagatatttctggatattgtcataaaacaatttagtgaatttatcatcgtccacttgaatctgtggttcattacgtcttaactcttcatatttagaaatgaggctgatgagttccatatttgaaaagttttcatcactacttagttttttgatagcttcaagccagagttgtctttttctatctactctcatacaaccaataaatgctgaaatgaattctaagcggagatcgcctagtgattttaaactattgctggcagcattcttgagtccaatataaaagtattgtgtaccttttgctgggtcaggttgttctttaggaggagtaaaaggatcaaatgcactaaacgaaactgaaacaagcgatcgaaaatatccctttgggattcttgactcgataagtctattattttcagagaaaaaatattcattgttttctgggttggtgattgcaccaatcattccattcaaaattgttgttttaccacacccattccgcccgataaaagcatgaatgttcgtgctgggcatagaattaaccgtcacctcaaaaggtatagttaaatcactgaatccgggagcactttttctattaaatgaaaagtggaaatctgacaattctggcaaaccatttaacacacgtgcgaactgtccatgaatttctgaaagagttacccctctaagtaatgaggtgttaaggacgctttcattttcaatgtcggctaatcgatttggccatactactaaatcctgaatagctttaagaaggttatgtttaaaaccatcgcttaatttgctgagattaacatagtagtcaatgctttcacctaaggaaaaaaacatttcagggagttgactgaattttttatctattaatgaataagtgcttacttcttctttttgacctacaaaaccaattttaacatttccgatatcgcatttttcaccatgctcatcaaagacagtaagataaaacattgtaacaaaggaatagtcattccaaccatctgctcgtaggaatgccttatttttttctactgcaggaatatacccgcctctttcaataacactaaactccaacatatagtaacccttaattttattaaaataaccgcaatttatttggcggcaacacaggatctctcttttaagttactctctattacatacgttttccatctaaaaattagtagtattgaacttaacggggcatcgtattgtagttttccatatttagctttctgcttccttttggataacccactgttattcatgttgcatggtgcactgtttataccaacgatatagtctattaatgcatatatagtatcgccgaacgattagctcttcaggcttctgaagaagcgtttcaagtactaataagccgatagatagccacggacttcgtagccatttttcataagtgttaacttccgctcctcgctcataacagacattcactacagttatggcggaaaggtatgcatgctgggtgtggggaagtcgtgaaagaaaagaagtcagctgcgtcgtttgacatcactgctatcttcttactggttatgcaggtcgtagtgggtggcacacaa

SEQ ID NO: 11 - DNA, 29 bp, Artificial Sequence
  Synthetic
tctttccctacacgatccgacggtagtgt